European Patent Application EP 4 226 972 A1, published August 16, 2023. Title: antibody and chimeric antigen receptor (CAR) binding to CD70, and application thereof. Applicant: Nanjing IASO Biotechnology Co., Ltd. The sequence listing filed with the application follows.

SEQUENCE LISTING (94 sequences)

SEQ ID NO: 1 - DNA, 63 bp, Artificial
  CD8a signal nucleic acid sequence
atggccctgcctgtgacagctctgctcctccctctggccctgctgctccatgccgccagaccc

SEQ ID NO: 2 - DNA, 63 bp, Artificial
  CD8a signal nucleic acid sequence
atggccctacctgtgacagccctactgttacccctggccctccttctgcatgctgctagacct

SEQ ID NO: 3 - protein, 21 aa, Artificial
  CD8a signal protein sequence
MALPVTALLLPLALLLHAARP

SEQ ID NO: 4 - DNA, 165 bp, Artificial
  CD8a hinge nucleic acid sequence
ttcgtgcccgtgttcctgcccgccaaacctactactacccctgcacctaggcctcccaccccagccccaacaatcgccagccagcctctgtctctgcggcccgaagcctgtagacctgctgccggcggagccgtgcacaccagaggcctggacttcgcctgcgac

SEQ ID NO: 5 - DNA, 165 bp, Artificial
  CD8a hinge nucleic acid sequence
tttgtgcctgtatttctgcctgccaagcccaccacaacacctgcccctagaccacccacccctgcccccaccattgcttctcagccccttagcttaagacctgaagcctgtagacctgctgctgggggggctgtgcacacaagaggcctggactttgcctgtgac

SEQ ID NO: 6 - protein, 55 aa, Artificial
  CD8a hinge protein sequence
FVPVFLPAKPTTTPAPRPPTPAPTIASQPLSLRPEACRPAAGGAVHTRGLDFACD

SEQ ID NO: 7 - DNA, 84 bp, Artificial
  CD8a TM nucleic acid sequence
atctacatctgggcccctctggccggcacctgtggcgtgctgctgctgagcctggtgatcaccctgtactgcaaccaccggaac

SEQ ID NO: 8 - DNA, 84 bp, Artificial
  CD8a TM nucleic acid sequence
atctacatctgggcccccctggctggcacctgtggggtgctgctgctgagcctggtgatcaccctgtactgcaaccacagaaac

SEQ ID NO: 9 - protein, 28 aa, Artificial
  CD8a TM protein sequence
IYIWAPLAGTCGVLLLSLVITLYCNHRN

SEQ ID NO: 10 - DNA, 126 bp, Artificial
  4-1BB intracellular domain nucleic acid sequence
aaacggggcagaaagaaactcctgtatatattcaaacaaccatttatgagaccagtacaaactactcaagaggaagatggctgtagctgccgatttccagaagaagaagaaggaggatgtgaactg

SEQ ID NO: 11 - DNA, 126 bp, Artificial
  4-1BB intracellular domain nucleic acid sequence
aagagaggcagaaagaagctgctgtacatcttcaagcagcccttcatgagacctgtgcagaccacccaagaggaggatggctgcagctgcagattccctgaggaggaggaggggggctgtgagctg

SEQ ID NO: 12 - protein, 42 aa, Artificial
  4-1BB intracellular domain protein sequence
KRGRKKLLYIFKQPFMRPVQTTQEEDGCSCRFPEEEEGGCEL

SEQ ID NO: 13 - DNA, 336 bp, Artificial
  CD3z intracellular signaling domain nucleic acid sequence
agagtgaagttcagcagatccgccgacgcccctgcctaccagcagggacagaaccagctgtacaacgagctgaacctgggcagacgggaagagtacgacgtgctggacaagcggagaggccgggaccccgagatgggcggaaagcccagacggaagaacccccaggaaggcctgtataacgaactgcagaaagacaagatggccgaggcctacagcgagatcggcatgaagggcgagcggaggcgcggcaagggccacgatggcctgtaccagggcctgagcaccgccaccaaggacacctacgacgccctgcacatgcaggccctgccccccaga

SEQ ID NO: 14 - DNA, 336 bp, Artificial
  CD3z intracellular signaling domain nucleic acid sequence
agagtgaagttcagcagatctgctgatgcccctgcctatcagcaagggcagaatcagctgtacaatgagctgaatctgggcagaagagaggagtatgatgtgctggacaagagaagaggcagagaccctgagatggggggcaagcctagaagaaagaacccccaagagggcctgtataatgagctgcagaaggacaagatggctgaggcctactctgagattggcatgaagggggagagaagaagaggcaagggccatgatggcctgtaccaaggcctgagcacagccaccaaggacacctatgatgccctacacatgcaagctctgcctcctaga

SEQ ID NO: 15 - protein, 112 aa, Artificial
  CD3z intracellular signaling domain protein sequence
RVKFSRSADAPAYQQGQNQLYNELNLGRREEYDVLDKRRGRDPEMGGKPRRKNPQEGLYNELQKDKMAEAYSEIGMKGERRRGKGHDGLYQGLSTATKDTYDALHMQALPPR

SEQ ID NO: 16 - DNA, 54 bp, Artificial
  Cleaving peptide T2A nucleic acid sequence
gagggaaggggcagcttattaacatgtggcgatgtggaagagaaccccggtccc

SEQ ID NO: 17 - DNA, 54 bp, Artificial
  Cleaving peptide T2A nucleic acid sequence
gaaggaaggggcagcctactgacctgtggggatgtggaggagaaccctggcccc

SEQ ID NO: 18 - protein, 18 aa, Artificial
  Cleaving peptide T2A protein sequence
EGRGSLLTCGDVEENPGP

SEQ ID NO: 19 - DNA, 66 bp, Artificial
  CSF2RA signal nucleic acid sequence
atgctgctgctcgtgacctctttactgttatgtgagctgccccaccccgcttttttactgatccct

SEQ ID NO: 20 - DNA, 66 bp, Artificial
  CSF2RA signal nucleic acid sequence
atgttgctattagtaaccagcctgctgctgtgtgagctgccccaccctgccttcctgttaatccca

SEQ ID NO: 21 - protein, 22 aa, Artificial
  CSF2RA signal protein sequence
MLLLVTSLLLCELPHPAFLLIP

SEQ ID NO: 22 - DNA, 1005 bp, Artificial
  tEGFR nucleic acid sequence
cgtaaggtgtgtaacggaatcggcattggcgagttcaaggactctttaagcatcaacgccacaaacatcaagcacttcaagaattgtacctccatcagcggcgatttacacattctccccgtggcttttcgtggcgattccttcacccacaccccccctctggacccccaagagctggacattttaaaaaccgtgaaggagatcaccggctttctgctgatccaagcttggcccgagaatcgtaccgacctccacgccttcgagaatttagagattattcgtggaaggaccaagcagcacggccagttctctttagccgtcgtgtctttaaacattaccagcctcggtttaaggtctttaaaggagattagcgacggcgacgtgatcatctccggcaacaagaacctctgctacgccaacaccatcaactggaagaagctgttcggaaccagcggccaaaagaccaagatcatcagcaatcgtggagagaactcttgtaaggccactggtcaagtttgccacgccctctgtagccccgaaggatgttggggccccgagcctagggactgtgttagctgcagaaacgtgagcagaggcagagagtgtgtggacaaatgcaatttactggaaggagagcctagggagttcgtggagaacagcgaatgtatccagtgccaccccgagtgtttacctcaagccatgaacatcacttgtaccggaaggggccccgataactgcatccaatgcgcccactacatcgacggaccccactgcgtgaaaacttgtcccgccggagtgatgggagagaataacactttagtgtggaagtacgccgacgctggccacgtctgccatctgtgccaccccaactgtacctacggctgcactggtcccggtttagagggatgtcctaccaacggccccaagatcccctccatcgccaccggaatggtgggcgctctgttattactgctggtggtggctctgggcatcggtttattcatg

SEQ ID NO: 23 - DNA, 1005 bp, Artificial
  tEGFR nucleic acid sequence
cgaaaggtatgtaatggcattggcattggggagtttaaggacagcctgagcatcaatgccaccaacatcaagcacttcaagaactgcacaagcatcagtggggacttgcacatcctgcctgtggccttcagaggggacagcttcacccacaccccccccctggacccccaagagctggacatcctgaagacagtgaaggagatcactggcttcttgctgatccaagcctggcctgagaacagaacagacctgcatgcctttgagaacctggagatcatcagaggcagaaccaagcagcatgggcagttcagcctggctgtggtgagcctgaacatcacaagcctgggcctgagaagcttaaaggagatctctgatggggatgtgatcatctctggcaacaagaacctgtgctatgccaacaccatcaactggaagaagctgtttggcacctctgggcagaagaccaagatcatcagcaacagaggggagaactcctgtaaggccactggccaagtgtgtcatgccctatgcagccctgaggggtgctggggccctgagcctagagactgtgtgagctgcagaaatgtgagcagaggcagagagtgtgtggacaagtgcaacctgctggagggggagcctagagagtttgtggagaactctgagtgtattcagtgtcatcctgagtgcctgccccaagccatgaacatcacctgcactggcagaggccctgacaactgcattcagtgtgcccactacattgatggcccccactgtgtgaagacctgccctgctggggtgatgggggagaacaacaccctggtgtggaagtatgctgatgctggccatgtgtgtcacctgtgccatcccaactgcacctatggctgcactggccctggcctggagggctgccccaccaatggtcccaagattcctagcattgccactggcatggtgggggccctgctcctacttctggtggttgccctgggcattggcctgttcatg

SEQ ID NO: 24 - protein, 335 aa, Artificial
  tEGFR protein sequence
RKVCNGIGIGEFKDSLSINATNIKHFKNCTSISGDLHILPVAFRGDSFTHTPPLDPQELDILKTVKEITGFLLIQAWPENRTDLHAFENLEIIRGRTKQHGQFSLAVVSLNITSLGLRSLKEISDGDVIISGNKNLCYANTINWKKLFGTSGQKTKIISNRGENSCKATGQVCHALCSPEGCWGPEPRDCVSCRNVSRGRECVDKCNLLEGEPREFVENSECIQCHPECLPQAMNITCTGRGPDNCIQCAHYIDGPHCVKTCPAGVMGENNTLVWKYADAGHVCHLCHPNCTYGCTGPGLEGCPTNGPKIPSIATGMVGALLLLLVVALGIGLFM

SEQ ID NO: 25 - DNA, 759 bp, Artificial
  Scfv 06  nucleic acid sequence
caggctgtgctgactcagccaccctcagcgtctgcgacccccgggcagagggtctccatctcctgttcggggagcagctccaacatcggaaggaatactgttaattggtaccagcacctccctggaacggcccccaaactcctcatttatagtaatgatcatcggccctcaggggtccctgaccgattctctggctcccagtctggcacctcagcctccctggccatcagtgggctccagtctgaggatgaggctgattattactgtgcatcatgggatgacagcctgactggatgggtgttcggcggagggaccaaggtcaccgtcctaggttctagaggtggtggtggtagcggcggcggcggctctggtggtggtggatccctcgagatggcccaggtgcagctggtgcagtctggggctgaggtgaagaaggctgggtcctcgctgaaggtctcgtgcaaggctaatggaggcagtttcaccaactatcttatcaactgggtgcgccaggcccctggacaggggcttgagtggatgggagggatcatccctgtctatggaacaccaatctactcacagaaattccagggcagagtcacatttaccgcggacgagcccacgaggacagcctacatggaactgagcagcctgacatttgaggacacggccgtgtattattgtgtgagagaagacgaaggctacggtgacctttatctcgcctactggggacaggggaccctggtcaccgtctcctca

SEQ ID NO: 26 - protein, 253 aa, Artificial
  Scfv 06 protein sequence
QAVLTQPPSASATPGQRVSISCSGSSSNIGRNTVNWYQHLPGTAPKLLIYSNDHRPSGVPDRFSGSQSGTSASLAISGLQSEDEADYYCASWDDSLTGWVFGGGTKVTVLGSRGGGGSGGGGSGGGGSLEMAQVQLVQSGAEVKKAGSSLKVSCKANGGSFTNYLINWVRQAPGQGLEWMGGIIPVYGTPIYSQKFQGRVTFTADEPTRTAYMELSSLTFEDTAVYYCVREDEGYGDLYLAYWGQGTLVTVSS

SEQ ID NO: 27 - DNA, 369 bp, Artificial
  VH06 nucleic acid sequence
atggcccaggtgcagctggtgcagtctggggctgaggtgaagaaggctgggtcctcgctgaaggtctcgtgcaaggctaatggaggcagtttcaccaactatcttatcaactgggtgcgccaggcccctggacaggggcttgagtggatgggagggatcatccctgtctatggaacaccaatctactcacagaaattccagggcagagtcacatttaccgcggacgagcccacgaggacagcctacatggaactgagcagcctgacatttgaggacacggccgtgtattattgtgtgagagaagacgaaggctacggtgacctttatctcgcctactggggacaggggaccctggtcaccgtctcctca

SEQ ID NO: 28 - protein, 123 aa, Artificial
  VH06 protein sequence
MAQVQLVQSGAEVKKAGSSLKVSCKANGGSFTNYLINWVRQAPGQGLEWMGGIIPVYGTPIYSQKFQGRVTFTADEPTRTAYMELSSLTFEDTAVYYCVREDEGYGDLYLAYWGQGTLVTVSS

SEQ ID NO: 29 - DNA, 333 bp, Artificial
  VL06 nucleic acid sequence
caggctgtgctgactcagccaccctcagcgtctgcgacccccgggcagagggtctccatctcctgttcggggagcagctccaacatcggaaggaatactgttaattggtaccagcacctccctggaacggcccccaaactcctcatttatagtaatgatcatcggccctcaggggtccctgaccgattctctggctcccagtctggcacctcagcctccctggccatcagtgggctccagtctgaggatgaggctgattattactgtgcatcatgggatgacagcctgactggatgggtgttcggcggagggaccaaggtcaccgtcctaggt

SEQ ID NO: 30 - protein, 111 aa, Artificial
  VL06 protein sequence
QAVLTQPPSASATPGQRVSISCSGSSSNIGRNTVNWYQHLPGTAPKLLIYSNDHRPSGVPDRFSGSQSGTSASLAISGLQSEDEADYYCASWDDSLTGWVFGGGTKVTVLG

SEQ ID NO: 31 - DNA, 369 bp, Artificial
  VHH 09 nucleic acid sequence
gaagttcagctgctggaaagcggtggtggtctggttcagcctggtggtagcctgcgtctgagctgtgcagcaagcggttttacctttaacatcgatgccatgggttgggttcgtcaggcacctggtaaaggtctggaatgggttagcagcatcagcagcagcggcggcaccacctattatgcagatagcgttaaaggtcgttttaccattagccgtgataacagcaaaaataccctgtacctgcagatgaatagtctgcgtgcagaggataccgcagtgtattattgtgcgcgctctcgttactctgttccggacggtcgtggttcttacgatgtttggggtcaaggtactctggtgaccgtctcctca

SEQ ID NO: 32 - DNA, 369 bp, Artificial
  VHH 09 nucleic acid sequence
gaggtgcaacttcttgagtctggggggggcttggtgcagcctgggggcagtctgagactgagctgtgctgcctctggctttaccttcaacattgatgccatgggttgggtaagacaagcccctggcaagggtctggagtgggtgagcagcatcagctcttctgggggcactacctactatgctgactctgtgaagggcagattcaccatcagcagagacaacagcaagaacaccctgtacctgcaaatgaatagccttagggctgaggacacagctgtatactactgtgctagaagcagatactctgtgcctgatggcagaggcagctatgatgtgtggggccaagggaccttggtcacagtgagctct

SEQ ID NO: 33 - protein, 123 aa, Artificial
  VHH 09 protein sequence
EVQLLESGGGLVQPGGSLRLSCAASGFTFNIDAMGWVRQAPGKGLEWVSSISSSGGTTYYADSVKGRFTISRDNSKNTLYLQMNSLRAEDTAVYYCARSRYSVPDGRGSYDVWGQGTLVTVSS

SEQ ID NO: 34 - DNA, 363 bp, Artificial
  VHH13 nucleic acid sequence
gaagttcagctgctggaaagcggtggtggtctggttcagcctggtggtagcctgcgtctgagctgtgcagcaagcggttttacctttagcagcgaagccatgggttgggttcgtcaggcacctggtaaaggtctggaatgggttagcagcatcaacggcagcggccgcaacacctattatgcagatagcgttaaaggtcgttttaccattagccgtgataacagcaaaaataccctgtacctgcagatgaatagtctgcgtgcagaggataccgcagtgtattactgtgcgcgcaaacatggtgaatactacgactctggttacgatgtttggggtcaaggtactctggtgaccgtctcctca

SEQ ID NO: 35 - DNA, 363 bp, Artificial
  VHH13 nucleic acid sequence
gaggtgcagctactggaatctggggggggcttagttcagcctggtggtagccttagattaagctgtgctgcatctggcttcacctttagctctgaggccatgggttgggtaagacaagcccctggcaagggtctggagtgggtgagcagcatcaatggctctggcagaaacacctattatgctgattctgtgaagggcagattcaccatcagcagagacaacagcaagaacaccctgtacctgcagatgaacagcctcagagctgaagacacagctgtgtattattgtgctagaaaacatggggagtactatgactctggctatgatgtgtgggggcaaggcaccttagtgacagtgtcatct

SEQ ID NO: 36 - protein, 121 aa, Artificial
  VHH13 protein sequence
EVQLLESGGGLVQPGGSLRLSCAASGFTFSSEAMGWVRQAPGKGLEWVSSINGSGRNTYYADSVKGRFTISRDNSKNTLYLQMNSLRAEDTAVYYCARKHGEYYDSGYDVWGQGTLVTVSS

SEQ ID NO: 37 - DNA, 360 bp, Artificial
  VHH 20 nucleic acid sequence
gaagttcagctgctggaaagcggtggtggtctggttcagcctggtggtagcctgcgtctgagctgtgcagcaagcggttttacctttagcagctatgccatgggttgggttcgtcaggcacctggtaaaggtctggaatgggttagcagcatcagcggctatggcgaagaaacctattatgcagatagcgttaaaggtcgttttaccattagccgtgataacagcaaaaataccctgtacctgcagatgaatagtctgcgtgcagaggataccgcagtgtattattgtgcgcgcttctactaccgttactggaaagaattcgattactggggtcaaggtactctggtgaccgtctcctca

SEQ ID NO: 38 - DNA, 360 bp, Artificial
  VHH 20 nucleic acid sequence
gaggttcagctcctggaatctgggggggggctggttcaacctgggggctcactgaggctgagctgtgctgcctctggatttacctttagcagctatgccatgggttgggttcgtcaggcccctggcaagggcctggaatgggttagcagcattagtggttatggggaggagacctattatgctgactctgtgaaaggcagatttaccatcagcagagataatagcaaaaataccctgtacctacaaatgaacagcctgagagctgaggacacagctgtgtactactgtgctagattctactaccgttactggaaagagtttgactactggggccaaggcaccctggtgacagtgtcatcc

SEQ ID NO: 39 - protein, 120 aa, Artificial
  VHH20 protein sequence
EVQLLESGGGLVQPGGSLRLSCAASGFTFSSYAMGWVRQAPGKGLEWVSSISGYGEETYYADSVKGRFTISRDNSKNTLYLQMNSLRAEDTAVYYCARFYYRYWKEFDYWGQGTLVTVSS

SEQ ID NO: 40 - DNA, 378 bp, Artificial
  VHH21 nucleic acid sequence
gaagttcagctgctggaaagcggtggtggtctggttcagcctggtggtagcctgcgtctgagctgtgcagcaagcggttttacctttagcaactatgccatgggttgggttcgtcaggcacctggtaaaggtctggaatgggttagcagcatcaccggcctgggcggcaacatgtattatgcagatagcgttaaaggtcgttttaccattagccgtgataacagcaaaaataccctgtacctgcagatgaatagtctgcgtgcagaggataccgcagtgtattattgtgcgcgcatgtactactctcagggtgttaacaactactcttacccgtctactgatatctggggtcaaggtactctggtgaccgtctcctca

SEQ ID NO: 41 - DNA, 378 bp, Artificial
  VHH21 nucleic acid sequence
gaggtgcagctgctggagtctggggggggcttggttcaacctgggggaagcctgaggctgagctgtgctgcctctggattcaccttcagcaattatgccatggggtgggttagacaagcccctggcaagggcctggagtgggtgtcaagcatcactggcctggggggcaacatgtattatgctgactctgtgaaaggcagatttaccatctctagagacaatagcaaaaataccctctatctgcagatgaatagcctgagagctgaggacacagctgtgtactattgtgctagaatgtactacagccaaggggtgaacaactacagctaccctagtactgatatatggggccaaggtactctggtgaccgtctccagc

SEQ ID NO: 42 - protein, 126 aa, Artificial
  VHH21 protein sequence
EVQLLESGGGLVQPGGSLRLSCAASGFTFSNYAMGWVRQAPGKGLEWVSSITGLGGNMYYADSVKGRFTISRDNSKNTLYLQMNSLRAEDTAVYYCARMYYSQGVNNYSYPSTDIWGQGTLVTVSS

SEQ ID NO: 43 - DNA, 48 bp, Artificial
  Whitlow Linker nucleic acid sequence
ggcagcacctctggctctggcaagcctggctctggggagggctcaaca

SEQ ID NO: 44 - protein, 16 aa, Artificial
  Whitlow Linker protein sequence
GSTSGSGKPGSGEGST

SEQ ID NO: 45 - DNA, 1533 bp, Artificial
  pXL1416 CAR nucleic acid sequence
atggccctgcctgtgacagctctgctcctccctctggccctgctgctccatgccgccagaccccaggctgtgctgactcagccaccctcagcgtctgcgacccccgggcagagggtctccatctcctgttcggggagcagctccaacatcggaaggaatactgttaattggtaccagcacctccctggaacggcccccaaactcctcatttatagtaatgatcatcggccctcaggggtccctgaccgattctctggctcccagtctggcacctcagcctccctggccatcagtgggctccagtctgaggatgaggctgattattactgtgcatcatgggatgacagcctgactggatgggtgttcggcggagggaccaaggtcaccgtcctaggttctagaggtggtggtggtagcggcggcggcggctctggtggtggtggatccctcgagatggcccaggtgcagctggtgcagtctggggctgaggtgaagaaggctgggtcctcgctgaaggtctcgtgcaaggctaatggaggcagtttcaccaactatcttatcaactgggtgcgccaggcccctggacaggggcttgagtggatgggagggatcatccctgtctatggaacaccaatctactcacagaaattccagggcagagtcacatttaccgcggacgagcccacgaggacagcctacatggaactgagcagcctgacatttgaggacacggccgtgtattattgtgtgagagaagacgaaggctacggtgacctttatctcgcctactggggacaggggaccctggtcaccgtctcctcattcgtgcccgtgttcctgcccgccaaacctactactacccctgcacctaggcctcccaccccagccccaacaatcgccagccagcctctgtctctgcggcccgaagcctgtagacctgctgccggcggagccgtgcacaccagaggcctggacttcgcctgcgacatctacatctgggcccctctggccggcacctgtggcgtgctgctgctgagcctggtgatcaccctgtactgcaaccaccggaacaaacggggcagaaagaaactcctgtatatattcaaacaaccatttatgagaccagtacaaactactcaagaggaagatggctgtagctgccgatttccagaagaagaagaaggaggatgtgaactgagagtgaagttcagcagatccgccgacgcccctgcctaccagcagggacagaaccagctgtacaacgagctgaacctgggcagacgggaagagtacgacgtgctggacaagcggagaggccgggaccccgagatgggcggaaagcccagacggaagaacccccaggaaggcctgtataacgaactgcagaaagacaagatggccgaggcctacagcgagatcggcatgaagggcgagcggaggcgcggcaagggccacgatggcctgtaccagggcctgagcaccgccaccaaggacacctacgacgccctgcacatgcaggccctgccccccaga

SEQ ID NO: 46 - protein, 511 aa, Artificial
  pXL1416 CAR protein sequence
MALPVTALLLPLALLLHAARPQAVLTQPPSASATPGQRVSISCSGSSSNIGRNTVNWYQHLPGTAPKLLIYSNDHRPSGVPDRFSGSQSGTSASLAISGLQSEDEADYYCASWDDSLTGWVFGGGTKVTVLGSRGGGGSGGGGSGGGGSLEMAQVQLVQSGAEVKKAGSSLKVSCKANGGSFTNYLINWVRQAPGQGLEWMGGIIPVYGTPIYSQKFQGRVTFTADEPTRTAYMELSSLTFEDTAVYYCVREDEGYGDLYLAYWGQGTLVTVSSFVPVFLPAKPTTTPAPRPPTPAPTIASQPLSLRPEACRPAAGGAVHTRGLDFACDIYIWAPLAGTCGVLLLSLVITLYCNHRNKRGRKKLLYIFKQPFMRPVQTTQEEDGCSCRFPEEEEGGCELRVKFSRSADAPAYQQGQNQLYNELNLGRREEYDVLDKRRGRDPEMGGKPRRKNPQEGLYNELQKDKMAEAYSEIGMKGERRRGKGHDGLYQGLSTATKDTYDALHMQALPPR

SEQ ID NO: 47 - DNA, 1143 bp, Artificial
  pXL1394 CAR nucleic acid sequence
atggccctgcctgtgacagctctgctcctccctctggccctgctgctccatgccgccagacccgaagttcagctgctggaaagcggtggtggtctggttcagcctggtggtagcctgcgtctgagctgtgcagcaagcggttttacctttaacatcgatgccatgggttgggttcgtcaggcacctggtaaaggtctggaatgggttagcagcatcagcagcagcggcggcaccacctattatgcagatagcgttaaaggtcgttttaccattagccgtgataacagcaaaaataccctgtacctgcagatgaatagtctgcgtgcagaggataccgcagtgtattattgtgcgcgctctcgttactctgttccggacggtcgtggttcttacgatgtttggggtcaaggtactctggtgaccgtctcctcattcgtgcccgtgttcctgcccgccaaacctactactacccctgcacctaggcctcccaccccagccccaacaatcgccagccagcctctgtctctgcggcccgaagcctgtagacctgctgccggcggagccgtgcacaccagaggcctggacttcgcctgcgacatctacatctgggcccctctggccggcacctgtggcgtgctgctgctgagcctggtgatcaccctgtactgcaaccaccggaacaaacggggcagaaagaaactcctgtatatattcaaacaaccatttatgagaccagtacaaactactcaagaggaagatggctgtagctgccgatttccagaagaagaagaaggaggatgtgaactgagagtgaagttcagcagatccgccgacgcccctgcctaccagcagggacagaaccagctgtacaacgagctgaacctgggcagacgggaagagtacgacgtgctggacaagcggagaggccgggaccccgagatgggcggaaagcccagacggaagaacccccaggaaggcctgtataacgaactgcagaaagacaagatggccgaggcctacagcgagatcggcatgaagggcgagcggaggcgcggcaagggccacgatggcctgtaccagggcctgagcaccgccaccaaggacacctacgacgccctgcacatgcaggccctgccccccaga

SEQ ID NO: 48 - protein, 381 aa, Artificial
  pXL1394 CAR protein sequence
MALPVTALLLPLALLLHAARPEVQLLESGGGLVQPGGSLRLSCAASGFTFNIDAMGWVRQAPGKGLEWVSSISSSGGTTYYADSVKGRFTISRDNSKNTLYLQMNSLRAEDTAVYYCARSRYSVPDGRGSYDVWGQGTLVTVSSFVPVFLPAKPTTTPAPRPPTPAPTIASQPLSLRPEACRPAAGGAVHTRGLDFACDIYIWAPLAGTCGVLLLSLVITLYCNHRNKRGRKKLLYIFKQPFMRPVQTTQEEDGCSCRFPEEEEGGCELRVKFSRSADAPAYQQGQNQLYNELNLGRREEYDVLDKRRGRDPEMGGKPRRKNPQEGLYNELQKDKMAEAYSEIGMKGERRRGKGHDGLYQGLSTATKDTYDALHMQALPPR

SEQ ID NO: 49 - DNA, 1137 bp, Artificial
  pXL1398 CAR nucleic acid sequence
atggccctgcctgtgacagctctgctcctccctctggccctgctgctccatgccgccagacccgaagttcagctgctggaaagcggtggtggtctggttcagcctggtggtagcctgcgtctgagctgtgcagcaagcggttttacctttagcagcgaagccatgggttgggttcgtcaggcacctggtaaaggtctggaatgggttagcagcatcaacggcagcggccgcaacacctattatgcagatagcgttaaaggtcgttttaccattagccgtgataacagcaaaaataccctgtacctgcagatgaatagtctgcgtgcagaggataccgcagtgtattactgtgcgcgcaaacatggtgaatactacgactctggttacgatgtttggggtcaaggtactctggtgaccgtctcctcattcgtgcccgtgttcctgcccgccaaacctactactacccctgcacctaggcctcccaccccagccccaacaatcgccagccagcctctgtctctgcggcccgaagcctgtagacctgctgccggcggagccgtgcacaccagaggcctggacttcgcctgcgacatctacatctgggcccctctggccggcacctgtggcgtgctgctgctgagcctggtgatcaccctgtactgcaaccaccggaacaaacggggcagaaagaaactcctgtatatattcaaacaaccatttatgagaccagtacaaactactcaagaggaagatggctgtagctgccgatttccagaagaagaagaaggaggatgtgaactgagagtgaagttcagcagatccgccgacgcccctgcctaccagcagggacagaaccagctgtacaacgagctgaacctgggcagacgggaagagtacgacgtgctggacaagcggagaggccgggaccccgagatgggcggaaagcccagacggaagaacccccaggaaggcctgtataacgaactgcagaaagacaagatggccgaggcctacagcgagatcggcatgaagggcgagcggaggcgcggcaagggccacgatggcctgtaccagggcctgagcaccgccaccaaggacacctacgacgccctgcacatgcaggccctgccccccaga

SEQ ID NO: 50 - protein, 379 aa, Artificial
  pXL1398 CAR protein sequence
MALPVTALLLPLALLLHAARPEVQLLESGGGLVQPGGSLRLSCAASGFTFSSEAMGWVRQAPGKGLEWVSSINGSGRNTYYADSVKGRFTISRDNSKNTLYLQMNSLRAEDTAVYYCARKHGEYYDSGYDVWGQGTLVTVSSFVPVFLPAKPTTTPAPRPPTPAPTIASQPLSLRPEACRPAAGGAVHTRGLDFACDIYIWAPLAGTCGVLLLSLVITLYCNHRNKRGRKKLLYIFKQPFMRPVQTTQEEDGCSCRFPEEEEGGCELRVKFSRSADAPAYQQGQNQLYNELNLGRREEYDVLDKRRGRDPEMGGKPRRKNPQEGLYNELQKDKMAEAYSEIGMKGERRRGKGHDGLYQGLSTATKDTYDALHMQALPPR

SEQ ID NO: 51 - DNA, 1134 bp, Artificial
  pXL1423 CAR nucleic acid sequence
atggccctgcctgtgacagctctgctcctccctctggccctgctgctccatgccgccagacccgaagttcagctgctggaaagcggtggtggtctggttcagcctggtggtagcctgcgtctgagctgtgcagcaagcggttttacctttagcagctatgccatgggttgggttcgtcaggcacctggtaaaggtctggaatgggttagcagcatcagcggctatggcgaagaaacctattatgcagatagcgttaaaggtcgttttaccattagccgtgataacagcaaaaataccctgtacctgcagatgaatagtctgcgtgcagaggataccgcagtgtattattgtgcgcgcttctactaccgttactggaaagaattcgattactggggtcaaggtactctggtgaccgtctcctcattcgtgcccgtgttcctgcccgccaaacctactactacccctgcacctaggcctcccaccccagccccaacaatcgccagccagcctctgtctctgcggcccgaagcctgtagacctgctgccggcggagccgtgcacaccagaggcctggacttcgcctgcgacatctacatctgggcccctctggccggcacctgtggcgtgctgctgctgagcctggtgatcaccctgtactgcaaccaccggaacaaacggggcagaaagaaactcctgtatatattcaaacaaccatttatgagaccagtacaaactactcaagaggaagatggctgtagctgccgatttccagaagaagaagaaggaggatgtgaactgagagtgaagttcagcagatccgccgacgcccctgcctaccagcagggacagaaccagctgtacaacgagctgaacctgggcagacgggaagagtacgacgtgctggacaagcggagaggccgggaccccgagatgggcggaaagcccagacggaagaacccccaggaaggcctgtataacgaactgcagaaagacaagatggccgaggcctacagcgagatcggcatgaagggcgagcggaggcgcggcaagggccacgatggcctgtaccagggcctgagcaccgccaccaaggacacctacgacgccctgcacatgcaggccctgccccccaga

SEQ ID NO: 52 - protein, 378 aa, Artificial
  pXL1423 CAR protein sequence
MALPVTALLLPLALLLHAARPEVQLLESGGGLVQPGGSLRLSCAASGFTFSSYAMGWVRQAPGKGLEWVSSISGYGEETYYADSVKGRFTISRDNSKNTLYLQMNSLRAEDTAVYYCARFYYRYWKEFDYWGQGTLVTVSSFVPVFLPAKPTTTPAPRPPTPAPTIASQPLSLRPEACRPAAGGAVHTRGLDFACDIYIWAPLAGTCGVLLLSLVITLYCNHRNKRGRKKLLYIFKQPFMRPVQTTQEEDGCSCRFPEEEEGGCELRVKFSRSADAPAYQQGQNQLYNELNLGRREEYDVLDKRRGRDPEMGGKPRRKNPQEGLYNELQKDKMAEAYSEIGMKGERRRGKGHDGLYQGLSTATKDTYDALHMQALPPR

SEQ ID NO: 53 - DNA, 1152 bp, Artificial
  pXL1424 CAR nucleic acid sequence
atggccctgcctgtgacagctctgctcctccctctggccctgctgctccatgccgccagacccgaagttcagctgctggaaagcggtggtggtctggttcagcctggtggtagcctgcgtctgagctgtgcagcaagcggttttacctttagcaactatgccatgggttgggttcgtcaggcacctggtaaaggtctggaatgggttagcagcatcaccggcctgggcggcaacatgtattatgcagatagcgttaaaggtcgttttaccattagccgtgataacagcaaaaataccctgtacctgcagatgaatagtctgcgtgcagaggataccgcagtgtattattgtgcgcgcatgtactactctcagggtgttaacaactactcttacccgtctactgatatctggggtcaaggtactctggtgaccgtctcctcattcgtgcccgtgttcctgcccgccaaacctactactacccctgcacctaggcctcccaccccagccccaacaatcgccagccagcctctgtctctgcggcccgaagcctgtagacctgctgccggcggagccgtgcacaccagaggcctggacttcgcctgcgacatctacatctgggcccctctggccggcacctgtggcgtgctgctgctgagcctggtgatcaccctgtactgcaaccaccggaacaaacggggcagaaagaaactcctgtatatattcaaacaaccatttatgagaccagtacaaactactcaagaggaagatggctgtagctgccgatttccagaagaagaagaaggaggatgtgaactgagagtgaagttcagcagatccgccgacgcccctgcctaccagcagggacagaaccagctgtacaacgagctgaacctgggcagacgggaagagtacgacgtgctggacaagcggagaggccgggaccccgagatgggcggaaagcccagacggaagaacccccaggaaggcctgtataacgaactgcagaaagacaagatggccgaggcctacagcgagatcggcatgaagggcgagcggaggcgcggcaagggccacgatggcctgtaccagggcctgagcaccgccaccaaggacacctacgacgccctgcacatgcaggccctgccccccaga

SEQ ID NO: 54 - protein, 384 aa, Artificial
  pXL1424 CAR protein sequence
MALPVTALLLPLALLLHAARPEVQLLESGGGLVQPGGSLRLSCAASGFTFSNYAMGWVRQAPGKGLEWVSSITGLGGNMYYADSVKGRFTISRDNSKNTLYLQMNSLRAEDTAVYYCARMYYSQGVNNYSYPSTDIWGQGTLVTVSSFVPVFLPAKPTTTPAPRPPTPAPTIASQPLSLRPEACRPAAGGAVHTRGLDFACDIYIWAPLAGTCGVLLLSLVITLYCNHRNKRGRKKLLYIFKQPFMRPVQTTQEEDGCSCRFPEEEEGGCELRVKFSRSADAPAYQQGQNQLYNELNLGRREEYDVLDKRRGRDPEMGGKPRRKNPQEGLYNELQKDKMAEAYSEIGMKGERRRGKGHDGLYQGLSTATKDTYDALHMQALPPR

SEQ ID NO: 55 - DNA, 1545 bp, Artificial
  pXL1698 CAR nucleic acid sequence
atggccctacctgtgacagccctactgttacccctggccctccttctgcatgctgctagacctgaggtgcagctactggaatctggggggggcttagttcagcctggtggtagccttagattaagctgtgctgcatctggcttcacctttagctctgaggccatgggttgggtaagacaagcccctggcaagggtctggagtgggtgagcagcatcaatggctctggcagaaacacctattatgctgattctgtgaagggcagattcaccatcagcagagacaacagcaagaacaccctgtacctgcagatgaacagcctcagagctgaagacacagctgtgtattattgtgctagaaaacatggggagtactatgactctggctatgatgtgtgggggcaaggcaccttagtgacagtgtcatctggcagcacctctggctctggcaagcctggctctggggagggctcaacagaggttcagctcctggaatctgggggggggctggttcaacctgggggctcactgaggctgagctgtgctgcctctggatttacctttagcagctatgccatgggttgggttcgtcaggcccctggcaagggcctggaatgggttagcagcattagtggttatggggaggagacctattatgctgactctgtgaaaggcagatttaccatcagcagagataatagcaaaaataccctgtacctacaaatgaacagcctgagagctgaggacacagctgtgtactactgtgctagattctactaccgttactggaaagagtttgactactggggccaaggcaccctggtgacagtgtcatcctttgtgcctgtatttctgcctgccaagcccaccacaacacctgcccctagaccacccacccctgcccccaccattgcttctcagccccttagcttaagacctgaagcctgtagacctgctgctgggggggctgtgcacacaagaggcctggactttgcctgtgacatctacatctgggcccccctggctggcacctgtggggtgctgctgctgagcctggtgatcaccctgtactgcaaccacagaaacaagagaggcagaaagaagctgctgtacatcttcaagcagcccttcatgagacctgtgcagaccacccaagaggaggatggctgcagctgcagattccctgaggaggaggaggggggctgtgagctgagagtgaagttcagcagatctgctgatgcccctgcctatcagcaagggcagaatcagctgtacaatgagctgaatctgggcagaagagaggagtatgatgtgctggacaagagaagaggcagagaccctgagatggggggcaagcctagaagaaagaacccccaagagggcctgtataatgagctgcagaaggacaagatggctgaggcctactctgagattggcatgaagggggagagaagaagaggcaagggccatgatggcctgtaccaaggcctgagcacagccaccaaggacacctatgatgccctacacatgcaagctctgcctcctaga

SEQ ID NO: 56 - protein, 513 aa, Artificial
  pXL1698 CAR protein sequence
MEFGLSWLFLVAILKGVQCEVQLLESGGGLVQPGGSLRLSCAASGFTFSSEAMGWVRQAPGKGLEWVSSINGSGRNTYYADSVKGRFTISRDNSKNTLYLQMNSLRAEDTAVYYCARKHGEYYDSGYDVWGQGTLVTVSSGSTSGSGKPGSGEGSTEVQLLESGGGLVQPGGSLRLSCAASGFTFSSYAMGWVRQAPGKGLEWVSSISGYGEETYYADSVKGRFTISRDNSKNTLYLQMNSLRAEDTAVYYCARFYYRYWKEFDYWGQGTLVTVSSFVPVFLPAKPTTTPAPRPPTPAPTIASQPLSLRPEACRPAAGGAVHTRGLDFACDIYIWAPLAGTCGVLLLSLVITLYCNHRNKRGRKKLLYIFKQPFMRPVQTTQEEDGCSCRFPEEEEGGCELRVKFSRSADAPAYQQGQNQLYNELNLGRREEYDVLDKRRGRDPEMGGKPRRKNPQEGLYNELQKDKMAEAYSEIGMKGERRRGKGHDGLYQGLSTATKDTYDALHMQALPPR

SEQ ID NO: 57 - DNA, 1545 bp, Artificial
  pXL1700 CAR  nucleic acid sequence
atggccctacctgtgacagccctactgttacccctggccctccttctgcatgctgctagacctgaggttcagctcctggaatctgggggggggctggttcaacctgggggctcactgaggctgagctgtgctgcctctggatttacctttagcagctatgccatgggttgggttcgtcaggcccctggcaagggcctggaatgggttagcagcattagtggttatggggaggagacctattatgctgactctgtgaaaggcagatttaccatcagcagagataatagcaaaaataccctgtacctacaaatgaacagcctgagagctgaggacacagctgtgtactactgtgctagattctactaccgttactggaaagagtttgactactggggccaaggcaccctggtgacagtgtcatccggcagcacctctggctctggcaagcctggctctggggagggctcaacagaggtgcagctactggaatctggggggggcttagttcagcctggtggtagccttagattaagctgtgctgcatctggcttcacctttagctctgaggccatgggttgggtaagacaagcccctggcaagggtctggagtgggtgagcagcatcaatggctctggcagaaacacctattatgctgattctgtgaagggcagattcaccatcagcagagacaacagcaagaacaccctgtacctgcagatgaacagcctcagagctgaagacacagctgtgtattattgtgctagaaaacatggggagtactatgactctggctatgatgtgtgggggcaaggcaccttagtgacagtgtcatcttttgtgcctgtatttctgcctgccaagcccaccacaacacctgcccctagaccacccacccctgcccccaccattgcttctcagccccttagcttaagacctgaagcctgtagacctgctgctgggggggctgtgcacacaagaggcctggactttgcctgtgacatctacatctgggcccccctggctggcacctgtggggtgctgctgctgagcctggtgatcaccctgtactgcaaccacagaaacaagagaggcagaaagaagctgctgtacatcttcaagcagcccttcatgagacctgtgcagaccacccaagaggaggatggctgcagctgcagattccctgaggaggaggaggggggctgtgagctgagagtgaagttcagcagatctgctgatgcccctgcctatcagcaagggcagaatcagctgtacaatgagctgaatctgggcagaagagaggagtatgatgtgctggacaagagaagaggcagagaccctgagatggggggcaagcctagaagaaagaacccccaagagggcctgtataatgagctgcagaaggacaagatggctgaggcctactctgagattggcatgaagggggagagaagaagaggcaagggccatgatggcctgtaccaaggcctgagcacagccaccaaggacacctatgatgccctacacatgcaagctctgcctcctaga

SEQ ID NO: 58 - protein, 515 aa, Artificial
  pXL1700 CAR protein sequence
MALPVTALLLPLALLLHAARPEVQLLESGGGLVQPGGSLRLSCAASGFTFSSYAMGWVRQAPGKGLEWVSSISGYGEETYYADSVKGRFTISRDNSKNTLYLQMNSLRAEDTAVYYCARFYYRYWKEFDYWGQGTLVTVSSGSTSGSGKPGSGEGSTEVQLLESGGGLVQPGGSLRLSCAASGFTFSSEAMGWVRQAPGKGLEWVSSINGSGRNTYYADSVKGRFTISRDNSKNTLYLQMNSLRAEDTAVYYCARKHGEYYDSGYDVWGQGTLVTVSSFVPVFLPAKPTTTPAPRPPTPAPTIASQPLSLRPEACRPAAGGAVHTRGLDFACDIYIWAPLAGTCGVLLLSLVITLYCNHRNKRGRKKLLYIFKQPFMRPVQTTQEEDGCSCRFPEEEEGGCELRVKFSRSADAPAYQQGQNQLYNELNLGRREEYDVLDKRRGRDPEMGGKPRRKNPQEGLYNELQKDKMAEAYSEIGMKGERRRGKGHDGLYQGLSTATKDTYDALHMQALPPR

SEQ ID NO: 59 - DNA, 1563 bp, Artificial
  pXL1702 CAR  nucleic acid sequence
atggccctacctgtgacagccctactgttacccctggccctccttctgcatgctgctagacctgaggtgcagctactggaatctggggggggcttagttcagcctggtggtagccttagattaagctgtgctgcatctggcttcacctttagctctgaggccatgggttgggtaagacaagcccctggcaagggtctggagtgggtgagcagcatcaatggctctggcagaaacacctattatgctgattctgtgaagggcagattcaccatcagcagagacaacagcaagaacaccctgtacctgcagatgaacagcctcagagctgaagacacagctgtgtattattgtgctagaaaacatggggagtactatgactctggctatgatgtgtgggggcaaggcaccttagtgacagtgtcatctggcagcacctctggctctggcaagcctggctctggggagggctcaacagaggtgcagctgctggagtctggggggggcttggttcaacctgggggaagcctgaggctgagctgtgctgcctctggattcaccttcagcaattatgccatggggtgggttagacaagcccctggcaagggcctggagtgggtgtcaagcatcactggcctggggggcaacatgtattatgctgactctgtgaaaggcagatttaccatctctagagacaatagcaaaaataccctctatctgcagatgaatagcctgagagctgaggacacagctgtgtactattgtgctagaatgtactacagccaaggggtgaacaactacagctaccctagtactgatatatggggccaaggtactctggtgaccgtctccagctttgtgcctgtatttctgcctgccaagcccaccacaacacctgcccctagaccacccacccctgcccccaccattgcttctcagccccttagcttaagacctgaagcctgtagacctgctgctgggggggctgtgcacacaagaggcctggactttgcctgtgacatctacatctgggcccccctggctggcacctgtggggtgctgctgctgagcctggtgatcaccctgtactgcaaccacagaaacaagagaggcagaaagaagctgctgtacatcttcaagcagcccttcatgagacctgtgcagaccacccaagaggaggatggctgcagctgcagattccctgaggaggaggaggggggctgtgagctgagagtgaagttcagcagatctgctgatgcccctgcctatcagcaagggcagaatcagctgtacaatgagctgaatctgggcagaagagaggagtatgatgtgctggacaagagaagaggcagagaccctgagatggggggcaagcctagaagaaagaacccccaagagggcctgtataatgagctgcagaaggacaagatggctgaggcctactctgagattggcatgaagggggagagaagaagaggcaagggccatgatggcctgtaccaaggcctgagcacagccaccaaggacacctatgatgccctacacatgcaagctctgcctcctaga

SEQ ID NO: 60 - protein, 521 aa, Artificial
  pXL1702 CAR protein sequence
MALPVTALLLPLALLLHAARPEVQLLESGGGLVQPGGSLRLSCAASGFTFSSEAMGWVRQAPGKGLEWVSSINGSGRNTYYADSVKGRFTISRDNSKNTLYLQMNSLRAEDTAVYYCARKHGEYYDSGYDVWGQGTLVTVSSGSTSGSGKPGSGEGSTEVQLLESGGGLVQPGGSLRLSCAASGFTFSNYAMGWVRQAPGKGLEWVSSITGLGGNMYYADSVKGRFTISRDNSKNTLYLQMNSLRAEDTAVYYCARMYYSQGVNNYSYPSTDIWGQGTLVTVSSFVPVFLPAKPTTTPAPRPPTPAPTIASQPLSLRPEACRPAAGGAVHTRGLDFACDIYIWAPLAGTCGVLLLSLVITLYCNHRNKRGRKKLLYIFKQPFMRPVQTTQEEDGCSCRFPEEEEGGCELRVKFSRSADAPAYQQGQNQLYNELNLGRREEYDVLDKRRGRDPEMGGKPRRKNPQEGLYNELQKDKMAEAYSEIGMKGERRRGKGHDGLYQGLSTATKDTYDALHMQALPPR

SEQ ID NO: 61 - DNA, 1563 bp, Artificial
  pXL1704 CAR  nucleic acid sequence
atggccctacctgtgacagccctactgttacccctggccctccttctgcatgctgctagacctgaggtgcagctgctggagtctggggggggcttggttcaacctgggggaagcctgaggctgagctgtgctgcctctggattcaccttcagcaattatgccatggggtgggttagacaagcccctggcaagggcctggagtgggtgtcaagcatcactggcctggggggcaacatgtattatgctgactctgtgaaaggcagatttaccatctctagagacaatagcaaaaataccctctatctgcagatgaatagcctgagagctgaggacacagctgtgtactattgtgctagaatgtactacagccaaggggtgaacaactacagctaccctagtactgatatatggggccaaggtactctggtgaccgtctccagcggcagcacctctggctctggcaagcctggctctggggagggctcaacagaggtgcagctactggaatctggggggggcttagttcagcctggtggtagccttagattaagctgtgctgcatctggcttcacctttagctctgaggccatgggttgggtaagacaagcccctggcaagggtctggagtgggtgagcagcatcaatggctctggcagaaacacctattatgctgattctgtgaagggcagattcaccatcagcagagacaacagcaagaacaccctgtacctgcagatgaacagcctcagagctgaagacacagctgtgtattattgtgctagaaaacatggggagtactatgactctggctatgatgtgtgggggcaaggcaccttagtgacagtgtcatcttttgtgcctgtatttctgcctgccaagcccaccacaacacctgcccctagaccacccacccctgcccccaccattgcttctcagccccttagcttaagacctgaagcctgtagacctgctgctgggggggctgtgcacacaagaggcctggactttgcctgtgacatctacatctgggcccccctggctggcacctgtggggtgctgctgctgagcctggtgatcaccctgtactgcaaccacagaaacaagagaggcagaaagaagctgctgtacatcttcaagcagcccttcatgagacctgtgcagaccacccaagaggaggatggctgcagctgcagattccctgaggaggaggaggggggctgtgagctgagagtgaagttcagcagatctgctgatgcccctgcctatcagcaagggcagaatcagctgtacaatgagctgaatctgggcagaagagaggagtatgatgtgctggacaagagaagaggcagagaccctgagatggggggcaagcctagaagaaagaacccccaagagggcctgtataatgagctgcagaaggacaagatggctgaggcctactctgagattggcatgaagggggagagaagaagaggcaagggccatgatggcctgtaccaaggcctgagcacagccaccaaggacacctatgatgccctacacatgcaagctctgcctcctaga

SEQ ID NO: 62 - protein, 521 aa, Artificial
  pXL1704 CAR protein sequence
MALPVTALLLPLALLLHAARPEVQLLESGGGLVQPGGSLRLSCAASGFTFSNYAMGWVRQAPGKGLEWVSSITGLGGNMYYADSVKGRFTISRDNSKNTLYLQMNSLRAEDTAVYYCARMYYSQGVNNYSYPSTDIWGQGTLVTVSSGSTSGSGKPGSGEGSTEVQLLESGGGLVQPGGSLRLSCAASGFTFSSEAMGWVRQAPGKGLEWVSSINGSGRNTYYADSVKGRFTISRDNSKNTLYLQMNSLRAEDTAVYYCARKHGEYYDSGYDVWGQGTLVTVSSFVPVFLPAKPTTTPAPRPPTPAPTIASQPLSLRPEACRPAAGGAVHTRGLDFACDIYIWAPLAGTCGVLLLSLVITLYCNHRNKRGRKKLLYIFKQPFMRPVQTTQEEDGCSCRFPEEEEGGCELRVKFSRSADAPAYQQGQNQLYNELNLGRREEYDVLDKRRGRDPEMGGKPRRKNPQEGLYNELQKDKMAEAYSEIGMKGERRRGKGHDGLYQGLSTATKDTYDALHMQALPPR

SEQ ID NO: 63 - DNA, 1554 bp, Artificial
  pXL1748 CAR  nucleic acid sequence
atggccctacctgtgacagccctactgttacccctggccctccttctgcatgctgctagacctgaggtgcaacttcttgagtctggggggggcttggtgcagcctgggggcagtctgagactgagctgtgctgcctctggctttaccttcaacattgatgccatgggttgggtaagacaagcccctggcaagggtctggagtgggtgagcagcatcagctcttctgggggcactacctactatgctgactctgtgaagggcagattcaccatcagcagagacaacagcaagaacaccctgtacctgcaaatgaatagccttagggctgaggacacagctgtatactactgtgctagaagcagatactctgtgcctgatggcagaggcagctatgatgtgtggggccaagggaccttggtcacagtgagctctggcagcacctctggctctggcaagcctggctctggggagggctcaacagaggtgcagctactggaatctggggggggcttagttcagcctggtggtagccttagattaagctgtgctgcatctggcttcacctttagctctgaggccatgggttgggtaagacaagcccctggcaagggtctggagtgggtgagcagcatcaatggctctggcagaaacacctattatgctgattctgtgaagggcagattcaccatcagcagagacaacagcaagaacaccctgtacctgcagatgaacagcctcagagctgaagacacagctgtgtattattgtgctagaaaacatggggagtactatgactctggctatgatgtgtgggggcaaggcaccttagtgacagtgtcatcttttgtgcctgtatttctgcctgccaagcccaccacaacacctgcccctagaccacccacccctgcccccaccattgcttctcagccccttagcttaagacctgaagcctgtagacctgctgctgggggggctgtgcacacaagaggcctggactttgcctgtgacatctacatctgggcccccctggctggcacctgtggggtgctgctgctgagcctggtgatcaccctgtactgcaaccacagaaacaagagaggcagaaagaagctgctgtacatcttcaagcagcccttcatgagacctgtgcagaccacccaagaggaggatggctgcagctgcagattccctgaggaggaggaggggggctgtgagctgagagtgaagttcagcagatctgctgatgcccctgcctatcagcaagggcagaatcagctgtacaatgagctgaatctgggcagaagagaggagtatgatgtgctggacaagagaagaggcagagaccctgagatggggggcaagcctagaagaaagaacccccaagagggcctgtataatgagctgcagaaggacaagatggctgaggcctactctgagattggcatgaagggggagagaagaagaggcaagggccatgatggcctgtaccaaggcctgagcacagccaccaaggacacctatgatgccctacacatgcaagctctgcctcctaga

SEQ ID NO: 64 - protein, 518 aa, Artificial
  pXL1748 CAR protein sequence
MALPVTALLLPLALLLHAARPEVQLLESGGGLVQPGGSLRLSCAASGFTFNIDAMGWVRQAPGKGLEWVSSISSSGGTTYYADSVKGRFTISRDNSKNTLYLQMNSLRAEDTAVYYCARSRYSVPDGRGSYDVWGQGTLVTVSSGSTSGSGKPGSGEGSTEVQLLESGGGLVQPGGSLRLSCAASGFTFSSEAMGWVRQAPGKGLEWVSSINGSGRNTYYADSVKGRFTISRDNSKNTLYLQMNSLRAEDTAVYYCARKHGEYYDSGYDVWGQGTLVTVSSFVPVFLPAKPTTTPAPRPPTPAPTIASQPLSLRPEACRPAAGGAVHTRGLDFACDIYIWAPLAGTCGVLLLSLVITLYCNHRNKRGRKKLLYIFKQPFMRPVQTTQEEDGCSCRFPEEEEGGCELRVKFSRSADAPAYQQGQNQLYNELNLGRREEYDVLDKRRGRDPEMGGKPRRKNPQEGLYNELQKDKMAEAYSEIGMKGERRRGKGHDGLYQGLSTATKDTYDALHMQALPPR

SEQ ID NO: 65 - DNA, 1554 bp, Artificial
  pXL1750 CAR  nucleic acid sequence
atggccctacctgtgacagccctactgttacccctggccctccttctgcatgctgctagacctgaggtgcagctactggaatctggggggggcttagttcagcctggtggtagccttagattaagctgtgctgcatctggcttcacctttagctctgaggccatgggttgggtaagacaagcccctggcaagggtctggagtgggtgagcagcatcaatggctctggcagaaacacctattatgctgattctgtgaagggcagattcaccatcagcagagacaacagcaagaacaccctgtacctgcagatgaacagcctcagagctgaagacacagctgtgtattattgtgctagaaaacatggggagtactatgactctggctatgatgtgtgggggcaaggcaccttagtgacagtgtcatctggcagcacctctggctctggcaagcctggctctggggagggctcaacagaggtgcaacttcttgagtctggggggggcttggtgcagcctgggggcagtctgagactgagctgtgctgcctctggctttaccttcaacattgatgccatgggttgggtaagacaagcccctggcaagggtctggagtgggtgagcagcatcagctcttctgggggcactacctactatgctgactctgtgaagggcagattcaccatcagcagagacaacagcaagaacaccctgtacctgcaaatgaatagccttagggctgaggacacagctgtatactactgtgctagaagcagatactctgtgcctgatggcagaggcagctatgatgtgtggggccaagggaccttggtcacagtgagctcttttgtgcctgtatttctgcctgccaagcccaccacaacacctgcccctagaccacccacccctgcccccaccattgcttctcagccccttagcttaagacctgaagcctgtagacctgctgctgggggggctgtgcacacaagaggcctggactttgcctgtgacatctacatctgggcccccctggctggcacctgtggggtgctgctgctgagcctggtgatcaccctgtactgcaaccacagaaacaagagaggcagaaagaagctgctgtacatcttcaagcagcccttcatgagacctgtgcagaccacccaagaggaggatggctgcagctgcagattccctgaggaggaggaggggggctgtgagctgagagtgaagttcagcagatctgctgatgcccctgcctatcagcaagggcagaatcagctgtacaatgagctgaatctgggcagaagagaggagtatgatgtgctggacaagagaagaggcagagaccctgagatggggggcaagcctagaagaaagaacccccaagagggcctgtataatgagctgcagaaggacaagatggctgaggcctactctgagattggcatgaagggggagagaagaagaggcaagggccatgatggcctgtaccaaggcctgagcacagccaccaaggacacctatgatgccctacacatgcaagctctgcctcctaga

SEQ ID NO: 66 - protein, 518 aa, Artificial
  pXL1750 CAR protein sequence
MALPVTALLLPLALLLHAARPEVQLLESGGGLVQPGGSLRLSCAASGFTFSSEAMGWVRQAPGKGLEWVSSINGSGRNTYYADSVKGRFTISRDNSKNTLYLQMNSLRAEDTAVYYCARKHGEYYDSGYDVWGQGTLVTVSSGSTSGSGKPGSGEGSTEVQLLESGGGLVQPGGSLRLSCAASGFTFNIDAMGWVRQAPGKGLEWVSSISSSGGTTYYADSVKGRFTISRDNSKNTLYLQMNSLRAEDTAVYYCARSRYSVPDGRGSYDVWGQGTLVTVSSFVPVFLPAKPTTTPAPRPPTPAPTIASQPLSLRPEACRPAAGGAVHTRGLDFACDIYIWAPLAGTCGVLLLSLVITLYCNHRNKRGRKKLLYIFKQPFMRPVQTTQEEDGCSCRFPEEEEGGCELRVKFSRSADAPAYQQGQNQLYNELNLGRREEYDVLDKRRGRDPEMGGKPRRKNPQEGLYNELQKDKMAEAYSEIGMKGERRRGKGHDGLYQGLSTATKDTYDALHMQALPPR

SEQ ID NO: 67 - DNA, 1569 bp, Artificial
  pXL1752 CAR  nucleic acid sequence
atggccctacctgtgacagccctactgttacccctggccctccttctgcatgctgctagacctgaggtgcaacttcttgagtctggggggggcttggtgcagcctgggggcagtctgagactgagctgtgctgcctctggctttaccttcaacattgatgccatgggttgggtaagacaagcccctggcaagggtctggagtgggtgagcagcatcagctcttctgggggcactacctactatgctgactctgtgaagggcagattcaccatcagcagagacaacagcaagaacaccctgtacctgcaaatgaatagccttagggctgaggacacagctgtatactactgtgctagaagcagatactctgtgcctgatggcagaggcagctatgatgtgtggggccaagggaccttggtcacagtgagctctggcagcacctctggctctggcaagcctggctctggggagggctcaacagaggtgcagctgctggagtctggggggggcttggttcaacctgggggaagcctgaggctgagctgtgctgcctctggattcaccttcagcaattatgccatggggtgggttagacaagcccctggcaagggcctggagtgggtgtcaagcatcactggcctggggggcaacatgtattatgctgactctgtgaaaggcagatttaccatctctagagacaatagcaaaaataccctctatctgcagatgaatagcctgagagctgaggacacagctgtgtactattgtgctagaatgtactacagccaaggggtgaacaactacagctaccctagtactgatatatggggccaaggtactctggtgaccgtctccagctttgtgcctgtatttctgcctgccaagcccaccacaacacctgcccctagaccacccacccctgcccccaccattgcttctcagccccttagcttaagacctgaagcctgtagacctgctgctgggggggctgtgcacacaagaggcctggactttgcctgtgacatctacatctgggcccccctggctggcacctgtggggtgctgctgctgagcctggtgatcaccctgtactgcaaccacagaaacaagagaggcagaaagaagctgctgtacatcttcaagcagcccttcatgagacctgtgcagaccacccaagaggaggatggctgcagctgcagattccctgaggaggaggaggggggctgtgagctgagagtgaagttcagcagatctgctgatgcccctgcctatcagcaagggcagaatcagctgtacaatgagctgaatctgggcagaagagaggagtatgatgtgctggacaagagaagaggcagagaccctgagatggggggcaagcctagaagaaagaacccccaagagggcctgtataatgagctgcagaaggacaagatggctgaggcctactctgagattggcatgaagggggagagaagaagaggcaagggccatgatggcctgtaccaaggcctgagcacagccaccaaggacacctatgatgccctacacatgcaagctctgcctcctaga

SEQ ID NO: 68 - protein, 523 aa, Artificial
  pXL1752 CAR protein sequence
MALPVTALLLPLALLLHAARPEVQLLESGGGLVQPGGSLRLSCAASGFTFNIDAMGWVRQAPGKGLEWVSSISSSGGTTYYADSVKGRFTISRDNSKNTLYLQMNSLRAEDTAVYYCARSRYSVPDGRGSYDVWGQGTLVTVSSGSTSGSGKPGSGEGSTEVQLLESGGGLVQPGGSLRLSCAASGFTFSNYAMGWVRQAPGKGLEWVSSITGLGGNMYYADSVKGRFTISRDNSKNTLYLQMNSLRAEDTAVYYCARMYYSQGVNNYSYPSTDIWGQGTLVTVSSFVPVFLPAKPTTTPAPRPPTPAPTIASQPLSLRPEACRPAAGGAVHTRGLDFACDIYIWAPLAGTCGVLLLSLVITLYCNHRNKRGRKKLLYIFKQPFMRPVQTTQEEDGCSCRFPEEEEGGCELRVKFSRSADAPAYQQGQNQLYNELNLGRREEYDVLDKRRGRDPEMGGKPRRKNPQEGLYNELQKDKMAEAYSEIGMKGERRRGKGHDGLYQGLSTATKDTYDALHMQALPPR

SEQ ID NO: 69 - DNA, 1569 bp, Artificial
  pXL1754 CAR  nucleic acid sequence
atggccctacctgtgacagccctactgttacccctggccctccttctgcatgctgctagacctgaggtgcagctgctggagtctggggggggcttggttcaacctgggggaagcctgaggctgagctgtgctgcctctggattcaccttcagcaattatgccatggggtgggttagacaagcccctggcaagggcctggagtgggtgtcaagcatcactggcctggggggcaacatgtattatgctgactctgtgaaaggcagatttaccatctctagagacaatagcaaaaataccctctatctgcagatgaatagcctgagagctgaggacacagctgtgtactattgtgctagaatgtactacagccaaggggtgaacaactacagctaccctagtactgatatatggggccaaggtactctggtgaccgtctccagcggcagcacctctggctctggcaagcctggctctggggagggctcaacagaggtgcaacttcttgagtctggggggggcttggtgcagcctgggggcagtctgagactgagctgtgctgcctctggctttaccttcaacattgatgccatgggttgggtaagacaagcccctggcaagggtctggagtgggtgagcagcatcagctcttctgggggcactacctactatgctgactctgtgaagggcagattcaccatcagcagagacaacagcaagaacaccctgtacctgcaaatgaatagccttagggctgaggacacagctgtatactactgtgctagaagcagatactctgtgcctgatggcagaggcagctatgatgtgtggggccaagggaccttggtcacagtgagctcttttgtgcctgtatttctgcctgccaagcccaccacaacacctgcccctagaccacccacccctgcccccaccattgcttctcagccccttagcttaagacctgaagcctgtagacctgctgctgggggggctgtgcacacaagaggcctggactttgcctgtgacatctacatctgggcccccctggctggcacctgtggggtgctgctgctgagcctggtgatcaccctgtactgcaaccacagaaacaagagaggcagaaagaagctgctgtacatcttcaagcagcccttcatgagacctgtgcagaccacccaagaggaggatggctgcagctgcagattccctgaggaggaggaggggggctgtgagctgagagtgaagttcagcagatctgctgatgcccctgcctatcagcaagggcagaatcagctgtacaatgagctgaatctgggcagaagagaggagtatgatgtgctggacaagagaagaggcagagaccctgagatggggggcaagcctagaagaaagaacccccaagagggcctgtataatgagctgcagaaggacaagatggctgaggcctactctgagattggcatgaagggggagagaagaagaggcaagggccatgatggcctgtaccaaggcctgagcacagccaccaaggacacctatgatgccctacacatgcaagctctgcctcctaga

SEQ ID NO: 70 - protein, 523 aa, Artificial
  pXL1754 CAR protein sequence
MALPVTALLLPLALLLHAARPEVQLLESGGGLVQPGGSLRLSCAASGFTFSNYAMGWVRQAPGKGLEWVSSITGLGGNMYYADSVKGRFTISRDNSKNTLYLQMNSLRAEDTAVYYCARMYYSQGVNNYSYPSTDIWGQGTLVTVSSGSTSGSGKPGSGEGSTEVQLLESGGGLVQPGGSLRLSCAASGFTFNIDAMGWVRQAPGKGLEWVSSISSSGGTTYYADSVKGRFTISRDNSKNTLYLQMNSLRAEDTAVYYCARSRYSVPDGRGSYDVWGQGTLVTVSSFVPVFLPAKPTTTPAPRPPTPAPTIASQPLSLRPEACRPAAGGAVHTRGLDFACDIYIWAPLAGTCGVLLLSLVITLYCNHRNKRGRKKLLYIFKQPFMRPVQTTQEEDGCSCRFPEEEEGGCELRVKFSRSADAPAYQQGQNQLYNELNLGRREEYDVLDKRRGRDPEMGGKPRRKNPQEGLYNELQKDKMAEAYSEIGMKGERRRGKGHDGLYQGLSTATKDTYDALHMQALPPR

SEQ ID NO: 71 - DNA, 9728 bp, Artificial
  Nucleic acid sequence of the GoldenGate backbone vector containing lethal gene ccdB
gccgctgatcttcagacctggaggaggagatatgagggacaattggagaagtgaattatataaatataaagtagtaaaaattgaaccattaggagtagcacccaccaaggcaaagagaagagtggtgcagagagaaaaaagagcagtgggaataggagctttgttccttgggttcttgggagcagcaggaagcactatgggcgcagcgtcaatgacgctgacggtacaggccagacaattattgtctggtatagtgcagcagcagaacaatttgctgagggctattgaggcgcaacagcatctgttgcaactcacagtctggggcatcaagcagctccaggcaagaatcctggctgtggaaagatacctaaaggatcaacagctcctggggatttggggttgctctggaaaactcatttgcaccactgctgtgccttggaatgctagttggagtaataaatctctggaacagatttggaatcacacgacctggatggagtgggacagagaaattaacaattacacaagcttaatacactccttaattgaagaatcgcaaaaccagcaagaaaagaatgaacaagaattattggaattagataaatgggcaagtttgtggaattggtttaacataacaaattggctgtggtatataaaattattcataatgatagtaggaggcttggtaggtttaagaatagtttttgctgtactttctatagtgaatagagttaggcagggatattcaccattatcgtttcagacccacctcccaaccccgaggggacccgacaggcccgaaggaatagaagaagaaggtggagagagagacagagacagatccattcgattagtgaacggatctcgacggtatcgcctttaaaagaaaaggggggattggggggtacagtgcaggggaaagaatagtagacataatagcaacagacatacaaactaaagaattacaaaaacaaattacaaaaattcaaaattttcgggtttattacagggacagcagagatccagtttatcgatcgtgaggctccggtgcccgtcagtgggcagagcgcacatcgcccacagtccccgagaagttggggggaggggtcggcaattgaaccggtgcctagagaaggtggcgcggggtaaactgggaaagtgatgtcgtgtactggctccgcctttttcccgagggtgggggagaaccgtatataagtgcagtagtcgccgtgaacgttctttttcgcaacgggtttgccgccagaacacaggtaagtgccgtgtgtggttcccgcgggcctggcctctttacgggttatggcccttgcgtgccttgaattacttccacctggctgcagtacgtgattcttgatcccgagcttcgggttggaagtgggtgggagagttcgaggccttgcgcttaaggagccccttcgcctcgtgcttgagttgaggcctggcctgggcgctggggccgccgcgtgcgaatctggtggcaccttcgcgcctgtctcgctgctttcgataagtctctagccatttaaaatttttgatgacctgctgcgacgctttttttctggcaagatagtcttgtaaatgcgggccaagatctgcacactggtatttcggtttttggggccgcgggcggcgacggggcccgtgcgtcccagcgcacatgttcggcgaggcggggcctgcgagcgcggccaccgagaatcggacgggggtagtctcaagctggccggcctgctctggtgcctggcctcgcgccgccgtgtatcgccccgccctgggcggcaaggctggcccggtcggcaccagttgcgtgagcggaaagatggccgcttcccggccctgctgcagggagctcaaaatggaggacgcggcgctcgggagagcgggcgggtgagtcacccacacaaaggaaaagggcctttccgtcctcagccgtcgcttcatgtgactccacggagtaccgggcgccgtccaggcacctcgattagttctcgagcttttggagtacgtcgtctttaggttggggggaggggttttatgcgatggagtttccccacactgagtgggtggagactgaagttaggccagcttggcacttgatgtaattctccttggaatttgccctttttgagtttggatcttggttcattctcaagcctcagacagtggttcaaagtttttttcttccatttcaggtgtcgtgaggaattagcttggtacgaattcctcgagactagttctagagcggccgcggatcgccgccaccatggccctgcctgtgacagctctgctcctccctctggccctgctgctccatgccgccagacccgagacgtgagaattaatacgactcactatagagggactggtgaaatgcagttcaaggtttacacctataaaagagagagccgctatcgcctgtttgtggatgtacagagtgatattattgacacgcccgggcgacggatggtgatccccctggccagtgcacgtctgctgtcagataaagtctcccgtgaactttacccggtggtgcatatcggggatgaaagctggcgcatgatgaccacccagatggtcagtgtgccggtctccgtcatcggagaagaagtggctgatctcagccaccgcgaaaatgacatcaaaaacgccattaatctgatgttctggggaatataacgtctcttcgtgcccgtgttcctgcccgccaaacctactactacccctgcacctaggcctcccaccccagccccaacaatcgccagccagcctctgtctctgcggcccgaagcctgtagacctgctgccggcggagccgtgcacaccagaggcctggacttcgcctgcgacatctacatctgggcccctctggccggcacctgtggcgtgctgctgctgagcctggtgatcaccctgtactgcaaccaccggaacaaacggggcagaaagaaactcctgtatatattcaaacaaccatttatgagaccagtacaaactactcaagaggaagatggctgtagctgccgatttccagaagaagaagaaggaggatgtgaactgagagtgaagttcagcagatccgccgacgcccctgcctaccagcagggacagaaccagctgtacaacgagctgaacctgggcagacgggaagagtacgacgtgctggacaagcggagaggccgggaccccgagatgggcggaaagcccagacggaagaacccccaggaaggcctgtataacgaactgcagaaagacaagatggccgaggcctacagcgagatcggcatgaagggcgagcggaggcgcggcaagggccacgatggcctgtaccagggcctgagcaccgccaccaaggacacctacgacgccctgcacatgcaggccctgccccccagaggatccggagagggaaggggcagcttattaacatgtggcgatgtggaagagaaccccggtcccatgctgctgctcgtgacctctttactgttatgtgagctgccccaccccgcttttttactgatccctcgtaaggtgtgtaacggaatcggcattggcgagttcaaggactctttaagcatcaacgccacaaacatcaagcacttcaagaattgtacctccatcagcggcgatttacacattctccccgtggcttttcgtggcgattccttcacccacaccccccctctggacccccaagagctggacattttaaaaaccgtgaaggagatcaccggctttctgctgatccaagcttggcccgagaatcgtaccgacctccacgccttcgagaatttagagattattcgtggaaggaccaagcagcacggccagttctctttagccgtcgtgtctttaaacattaccagcctcggtttaaggtctttaaaggagattagcgacggcgacgtgatcatctccggcaacaagaacctctgctacgccaacaccatcaactggaagaagctgttcggaaccagcggccaaaagaccaagatcatcagcaatcgtggagagaactcttgtaaggccactggtcaagtttgccacgccctctgtagccccgaaggatgttggggccccgagcctagggactgtgttagctgcagaaacgtgagcagaggcagagagtgtgtggacaaatgcaatttactggaaggagagcctagggagttcgtggagaacagcgaatgtatccagtgccaccccgagtgtttacctcaagccatgaacatcacttgtaccggaaggggccccgataactgcatccaatgcgcccactacatcgacggaccccactgcgtgaaaacttgtcccgccggagtgatgggagagaataacactttagtgtggaagtacgccgacgctggccacgtctgccatctgtgccaccccaactgtacctacggctgcactggtcccggtttagagggatgtcctaccaacggccccaagatcccctccatcgccaccggaatggtgggcgctctgttattactgctggtggtggctctgggcatcggtttattcatgtgaacgcgtctggaacaatcaacctctggattacaaaatttgtgaaagattgactggtattcttaactatgttgctccttttacgctatgtggatacgctgctttaatgcctttgtatcatgctattgcttcccgtatggctttcattttctcctccttgtataaatcctggttgctgtctctttatgaggagttgtggcccgttgtcaggcaacgtggcgtggtgtgcactgtgtttgctgacgcaacccccactggttggggcattgccaccacctgtcagctcctttccgggactttcgctttccccctccctattgccacggcggaactcatcgccgcctgccttgcccgctgctggacaggggctcggctgttgggcactgacaattccgtggtgttgtcggggaagctgacgtcctttccatggctgctcgcctgtgttgccacctggattctgcgcgggacgtccttctgctacgtcccttcggccctcaatccagcggaccttccttcccgcggcctgctgccggctctgcggcctcttccgcgtcttcgccttcgccctcagacgagtcggatctccctttgggccgcctccccgcctggaattaattctgcagtcgagacctagaaaaacatggagcaatcacaagtagcaatacagcagctaccaatgctgattgtgcctggctagaagcacaagaggaggaggaggtgggttttccagtcacacctcaggtacctttaagaccaatgacttacaaggcagctgtagatcttagccactttttaaaagaaaagaggggactggaagggctaattcactcccaacgaagacaagatatccttgatctgtggatctaccacacacaaggctacttccctgattagcagaactacacaccagggccaggggtcagatatccactgacctttggatggtgctacaagctagtaccagttgagccagataaggtagaagaggccaataaaggagagaacaccagcttgttacaccctgtgagcctgcatgggatggatgacccggagagagaagtgttagagtggaggtttgacagccgcctagcatttcatcacgtggcccgagagctgcatccggagtacttcaagaactgctgatatcgagcttgctacaagggactttccgctggggactttccagggaggcgtggcctgggcgggactggggagtggcgagccctcagatcctgcatataagcagctgctttttgcctgtactgggtctctctggttagaccagatctgagcctgggagctctctggctaactagggaacccactgcttaagcctcaataaagcttgccttgagtgcttcaagtagtgtgtgcccgtctgttgtgtgactctggtaactagagatccctcagacccttttagtcagtgtggaaaatctctagcagtagtagttcatgtcatcttattattcagtatttataacttgcaaagaaatgaatatcagagagtgagaggccttgacattgctagcgtttaccgtcgacctctagctagagcttggcgtaatcatggtcatagctgtttcctgtgtgaaattgttatccgctcacaattccacacaacatacgagccggaagcataaagtgtaaagcctggggtgcctaatgagtgagctaactcacattaattgcgttgcgctcactgcccgctttccagtcgggaaacctgtcgtgccagctgcattaatgaatcggccaacgcgcggggagaggcggtttgcgtattgggccgcttcctcgctcactgactcgctgcgctcggtcgttcggctgcggcgagcggtatcagctcactcaaaggcggtaatacggttatccacagaatcaggggataacgcaggaaagaacatgtgagcaaaaggccagcaaaaggccaggaaccgtaaaaaggccgcgttgctggcgtttttccataggctccgcccccctgacgagcatcacaaaaatcgacgctcaagtcagaggtggcgaaacccgacaggactataaagataccaggcgtttccccctggaagctccctcgtgcgctctcctgttccgaccctgccgcttaccggatacctgtccgcctttctcccttcgggaagcgtggcgctttctcatagctcacgctgtaggtatctcagttcggtgtaggtcgttcgctccaagctgggctgtgtgcacgaaccccccgttcagcccgaccgctgcgccttatccggtaactatcgtcttgagtccaacccggtaagacacgacttatcgccactggcagcagccactggtaacaggattagcagagcgaggtatgtaggcggtgctacagagttcttgaagtggtggcctaactacggctacactagaagaacagtatttggtatctgcgctctgctgaagccagttaccttcggaaaaagagttggtagctcttgatccggcaaacaaaccaccgctggtagcggtggtttttttgtttgcaagcagcagattacgcgcagaaaaaaaggatctcaagaagatcctttgatcttttctacggggtctgacgctcagtggaacgaaaactcacgttaagggattttggtcatgagattatcaaaaaggatcttcacctagatccttttaaattaaaaatgaagttttaaatcaatctaaagtatatatgagtaaacttggtctgacagttaccaatgcttaatcagtgaggcacctatctcagcgatctgtctatttcgttcatccatagttgcctgactccccgtcgtgtagataactacgatacgggagggcttaccatctggccccagtgctgcaatgataccgcgagacccacgctcaccggctccagatttatcagcaataaaccagccagccggaagggccgagcgcagaagtggtcctgcaactttatccgcctccatccagtctattaattgttgccgggaagctagagtaagtagttcgccagttaatagtttgcgcaacgttgttgccattgctacaggcatcgtggtgtcacgctcgtcgtttggtatggcttcattcagctccggttcccaacgatcaaggcgagttacatgatcccccatgttgtgcaaaaaagcggttagctccttcggtcctccgatcgttgtcagaagtaagttggccgcagtgttatcactcatggttatggcagcactgcataattctcttactgtcatgccatccgtaagatgcttttctgtgactggtgagtactcaaccaagtcattctgagaatagtgtatgcggcgaccgagttgctcttgcccggcgtcaatacgggataataccgcgccacatagcagaactttaaaagtgctcatcattggaaaacgttcttcggggcgaaaactctcaaggatcttaccgctgttgagatccagttcgatgtaacccactcgtgcacccaactgatcttcagcatcttttactttcaccagcgtttctgggtgagcaaaaacaggaaggcaaaatgccgcaaaaaagggaataagggcgacacggaaatgttgaatactcatactcttcctttttcaatattattgaagcatttatcagggttattgtctcatgagcggatacatatttgaatgtatttagaaaaataaacaaataggggttccgcgcacatttccccgaaaagtgccacctgacgtcgacggatcgggagatcaacttgtttattgcagcttataatggttacaaataaagcaatagcatcacaaatttcacaaataaagcatttttttcactgcattctagttgtggtttgtccaaactcatcaatgtatcttatcatgtctggatcaactggataactcaagctaaccaaaatcatcccaaacttcccaccccataccctattaccactgccaattacctgtggtttcatttactctaaacctgtgattcctctgaattattttcattttaaagaaattgtatttgttaaatatgtactacaaacttagtagttggaagggctaattcactcccaaagaagacaagatatccttgatctgtggatctaccacacacaaggctacttccctgattagcagaactacacaccagggccaggggtcagatatccactgacctttggatggtgctacaagctagtaccagttgagccagataaggtagaagaggccaataaaggagagaacaccagcttgttacaccctgtgagcctgcatgggatggatgacccggagagagaagtgttagagtggaggtttgacagccgcctagcatttcatcacgtggcccgagagctgcatccggagtacttcaagaactgctgatatcgagcttgctacaagggactttccgctggggactttccagggaggcgtggcctgggcgggactggggagtggcgagccctcagatcctgcatataagcagctgctttttgcctgtactgggtctctctggttagaccagatctgagcctgggagctctctggctaactagggaacccactgcttaagcctcaataaagcttgccttgagtgcttcaagtagtgtgtgcccgtctgttgtgtgactctggtaactagagatccctcagacccttttagtcagtgtggaaaatctctagcagtggcgcccgaacagggacttgaaagcgaaagggaaaccagaggagctctctcgacgcaggactcggcttgctgaagcgcgcacggcaagaggcgaggggcggcgactggtgagtacgccaaaaattttgactagcggaggctagaaggagagagatgggtgcgagagcgtcagtattaagcgggggagaattagatcgcgatgggaaaaaattcggttaaggccagggggaaagaaaaaatataaattaaaacatatagtatgggcaagcagggagctagaacgattcgcagttaatcctggcctgttagaaacatcagaaggctgtagacaaatactgggacagctacaaccatcccttcagacaggatcagaagaacttagatcattatataatacagtagcaaccctctattgtgtgcatcaaaggatagagataaaagacaccaaggaagctttagacaagatagagaaaacaaaagtaagaccaccgcacagcaagcggccg

SEQ ID NO: 72 - protein, 8 aa, Artificial
  amino acid sequence of HCDR1 of 06 antibody
GGSFTNYL

SEQ ID NO: 73 - protein, 8 aa, Artificial
  amino acid sequence of HCDR2 of 06 antibody
IIPVYGTP

SEQ ID NO: 74 - protein, 14 aa, Artificial
  amino acid sequence of HCDR3 of 06 antibody
VREDEGYGDLYLAY

SEQ ID NO: 75 - protein, 8 aa, Artificial
  amino acid sequence of LCDR1 of 06 antibody
SSNIGRNT

SEQ ID NO: 76 - protein, 3 aa, Artificial
  amino acid sequence of LCDR2 of 06 antibody
SND

SEQ ID NO: 77 - protein, 11 aa, Artificial
  amino acid sequence of LCDR3 of 06 antibody
ASWDDSLTGWV

SEQ ID NO: 78 - protein, 8 aa, Artificial
  amino acid sequence of HCDR1 of 09 antibody
GFTFNIDA

SEQ ID NO: 79 - protein, 8 aa, Artificial
  amino acid sequence of HCDR2 of 09 antibody
ISSSGGTT

SEQ ID NO: 80 - protein, 16 aa, Artificial
  amino acid sequence of HCDR3 of 09 antibody
ARSRYSVPDGRGSYDV

SEQ ID NO: 81 - protein, 8 aa, Artificial
  amino acid sequence of HCDR1 of 13 antibody
GFTFSSEA

SEQ ID NO: 82 - protein, 8 aa, Artificial
  amino acid sequence of HCDR2 of 13 antibody
INASGRNT

SEQ ID NO: 83 - protein, 14 aa, Artificial
  amino acid sequence of HCDR3 of 13 antibody
ARKHGEYYDSGYDV

SEQ ID NO: 84 - protein, 8 aa, Artificial
  amino acid sequence of HCDR1 of 20 antibody
GFTFSSYA

SEQ ID NO: 85 - protein, 8 aa, Artificial
  amino acid sequence of HCDR2 of 20 antibody
ISGYGEET

SEQ ID NO: 86 - protein, 13 aa, Artificial
  amino acid sequence of HCDR3 of 20 antibody
ARFYYRYWKEFDY

SEQ ID NO: 87 - protein, 8 aa, Artificial
  amino acid sequence of HCDR1 of 21 antibody
GFTFSNYA

SEQ ID NO: 88 - protein, 8 aa, Artificial
  amino acid sequence of HCDR2 of 21 antibody
ITGLGGNM

SEQ ID NO: 89 - protein, 19 aa, Artificial
  amino acid sequence of HCDR3 of 21 antibody
ARMYYSQGVNNYSYPSTDI

SEQ ID NO: 90 - DNA, 20 bp, Artificial
  sgRNA-1
gagcagcccgaaccctcctc

SEQ ID NO: 91 - DNA, 20 bp, Artificial
  sgRNA-2
ggaggagggttcgggctgct

SEQ ID NO: 92 - DNA, 20 bp, Artificial
  gRNA-3
atcaccaagcccgcgaccaa

SEQ ID NO: 93 - DNA, 20 bp, Artificial
  sgRNA-4
agcgctggatgcacaccacg

SEQ ID NO: 94 - DNA, 20 bp, Artificial
  sgRNA-5
gggcttggtgatctgcctcg